European Patent Application EP 4 582 550 A1, published July 9, 2025. Title: METHOD FOR TEMPLATE-FREE DE NOVO SYNTHESIS OF LONG-CHAIN NUCLEIC ACID, AND USE THEREOF. Applicant: SHANGHAI TYPING BIOSCIENCE CO., LTD. The sequence listing filed with the application follows.

SEQUENCE LISTING (129 sequences)

SEQ ID NO: 1 - DNA, 1856 bp, artificial series
  source 1..1856: mol_type = other DNA
atgaaaaggaactacattctggggctggacatcgggattacaagcgtggggtatgggattattgactatgaaacaagggacgtgatcgacgcaggcgtcagactgttcaaggaggccaacgtggaaaacaatgagggacggagaagcaagaggggagccaggcgcctgaaacgacggagaaggcacagaatccagagggtgaagaaactgctgttcgattacaacctgctgaccgaccattctgagctgagtggaattaatccttatgaagccagggtgaaaggcctgagtcagaagctgtcagaggaagagttttccgcagctctgctgcacctggctaagcgccgaggagtgcataacgtcaatgaggtggaagaggacaccggcaacgagctgtctacaaaggaacagatctcacgcaatagcaaagctctggaagagaagtatgtcgcagagctacagctggaacggctgaagaaagatggcgaggtgagagggtcaattaataggttcaagacaagcgactacgtcaaagaagccaagcagctgctgaaagtgcagaaggcttaccaccagctggatcagagcttcatcgatacttatatcgacctgctggagactcggagaacctactatgagggaccaggagaagggagccccttcggatggaaagacatcaaggaatggtacgagatgctgatgggacattgcacctattttccagaagagctgagaagcgtcaagtacgcttataacgcagatctgtacaacgccctgaatgacctgaacaacctggtcatcaccagggatgaaaacgagaaactggaatactatgagaagttccagatcatcgaaaacgtgtttaagcagaagaaaaagcctacactgaaacagattgctaaggagatcctggtcaacgaagaggacatcaagggctaccgggtgacaagcactggaaaaccagagttcaccaatctgaaagtgtatcacgatattaaggacatcacagcacggaaagaaatcattgagaacgccgaactgctggatcagattgctaagatcctgactatctaccagagttccgaggacatccaggaagagctgactaacctgaacagcgagctgacccaggaagagatcgaacagattagtaatctgaaggggtacaccggaacacacaacctgtccctgaaagctatcaatctgattctggatgagctgtggcatacaaacgacaatcagattgcaatctttaaccggctgaagctggtaccaaaaaaggtggacctgagtcagcagaaagagatcccaaccacactggtggacgatttcattctgtcacccgtggtcaagcggagcttcatccagagcatcaaagtgatcaacgccatcatcaagaagtacggcctgcccaatgatatcattatcgagctggctagggagaagaacagcaaggacgcacagaagatgatcaatgagatgcagaaacgaaaccggcagaccaatgaacgcattgaagagattatccgaactaccgggaaagagaacgcaaagtacctgattgaaaaaatcaagctgcacgatatgcaggagggaaagtgtctgtattctctggaggccatccccctggaggacctgctgaacaatccattcaactacgaggtcgatcatattatccccagaagcgtgtccttcgacaattcctttaacaacaaggtgctggtcaagcaggaagagaactctaaaaagggcaataggactcctttccagtacctgtctagttcagattccaagatctcttacgaaacctttaaaaagcacattctgaatctggccaaaggaaagggccgcatcag

SEQ ID NO: 2 - DNA, 19 bp, artificial series
  source 1..19: mol_type = other DNA
atgaaaaggaactacattc

SEQ ID NO: 3 - DNA, 29 bp, artificial series
  source 1..29: mol_type = other DNA
tggggctggacatcgggattacaagcgtg

SEQ ID NO: 4 - DNA, 29 bp, artificial series
  source 1..29: mol_type = other DNA
gggtatgggattattgactatgaaacaag

SEQ ID NO: 5 - DNA, 29 bp, artificial series
  source 1..29: mol_type = other DNA
ggacgtgatcgacgcaggcgtcagactgt

SEQ ID NO: 6 - DNA, 29 bp, artificial series
  source 1..29: mol_type = other DNA
tcaaggaggccaacgtggaaaacaatgag

SEQ ID NO: 7 - DNA, 29 bp, artificial series
  source 1..29: mol_type = other DNA
ggacggagaagcaagaggggagccaggcg

SEQ ID NO: 8 - DNA, 29 bp, artificial series
  source 1..29: mol_type = other DNA
cctgaaacgacggagaaggcacagaatcc

SEQ ID NO: 9 - DNA, 29 bp, artificial series
  source 1..29: mol_type = other DNA
agagggtgaagaaactgctgttcgattac

SEQ ID NO: 10 - DNA, 28 bp, artificial series
  source 1..28: mol_type = other DNA
aacctgctgaccgaccattctgagctga

SEQ ID NO: 11 - DNA, 30 bp, artificial series
  source 1..30: mol_type = other DNA
gtggaattaatccttatgaagccagggtga

SEQ ID NO: 12 - DNA, 29 bp, artificial series
  source 1..29: mol_type = other DNA
aaggcctgagtcagaagctgtcagaggaa

SEQ ID NO: 13 - DNA, 29 bp, artificial series
  source 1..29: mol_type = other DNA
gagttttccgcagctctgctgcacctggc

SEQ ID NO: 14 - DNA, 29 bp, artificial series
  source 1..29: mol_type = other DNA
taagcgccgaggagtgcataacgtcaatg

SEQ ID NO: 15 - DNA, 29 bp, artificial series
  source 1..29: mol_type = other DNA
aggtggaagaggacaccggcaacgagctg

SEQ ID NO: 16 - DNA, 29 bp, artificial series
  source 1..29: mol_type = other DNA
tctacaaaggaacagatctcacgcaatag

SEQ ID NO: 17 - DNA, 29 bp, artificial series
  source 1..29: mol_type = other DNA
caaagctctggaagagaagtatgtcgcag

SEQ ID NO: 18 - DNA, 29 bp, artificial series
  source 1..29: mol_type = other DNA
agctacagctggaacggctgaagaaagat

SEQ ID NO: 19 - DNA, 29 bp, artificial series
  source 1..29: mol_type = other DNA
ggcgaggtgagagggtcaattaataggtt

SEQ ID NO: 20 - DNA, 29 bp, artificial series
  source 1..29: mol_type = other DNA
caagacaagcgactacgtcaaagaagcca

SEQ ID NO: 21 - DNA, 29 bp, artificial series
  source 1..29: mol_type = other DNA
agcagctgctgaaagtgcagaaggcttac

SEQ ID NO: 22 - DNA, 28 bp, artificial series
  source 1..28: mol_type = other DNA
caccagctggatcagagcttcatcgata

SEQ ID NO: 23 - DNA, 29 bp, artificial series
  source 1..29: mol_type = other DNA
cttatatcgacctgctggagactcggaga

SEQ ID NO: 24 - DNA, 30 bp, artificial series
  source 1..30: mol_type = other DNA
acctactatgagggaccaggagaagggagc

SEQ ID NO: 25 - DNA, 29 bp, artificial series
  source 1..29: mol_type = other DNA
cccttcggatggaaagacatcaaggaatg

SEQ ID NO: 26 - DNA, 28 bp, artificial series
  source 1..28: mol_type = other DNA
gtacgagatgctgatgggacattgcacc

SEQ ID NO: 27 - DNA, 29 bp, artificial series
  source 1..29: mol_type = other DNA
tattttccagaagagctgagaagcgtcaa

SEQ ID NO: 28 - DNA, 30 bp, artificial series
  source 1..30: mol_type = other DNA
gtacgcttataacgcagatctgtacaacgc

SEQ ID NO: 29 - DNA, 29 bp, artificial series
  source 1..29: mol_type = other DNA
cctgaatgacctgaacaacctggtcatca

SEQ ID NO: 30 - DNA, 28 bp, artificial series
  source 1..28: mol_type = other DNA
ccagggatgaaaacgagaaactggaata

SEQ ID NO: 31 - DNA, 29 bp, artificial series
  source 1..29: mol_type = other DNA
ctatgagaagttccagatcatcgaaaacg

SEQ ID NO: 32 - DNA, 30 bp, artificial series
  source 1..30: mol_type = other DNA
tgtttaagcagaagaaaaagcctacactga

SEQ ID NO: 33 - DNA, 29 bp, artificial series
  source 1..29: mol_type = other DNA
aacagattgctaaggagatcctggtcaac

SEQ ID NO: 34 - DNA, 29 bp, artificial series
  source 1..29: mol_type = other DNA
gaagaggacatcaagggctaccgggtgac

SEQ ID NO: 35 - DNA, 28 bp, artificial series
  source 1..28: mol_type = other DNA
aagcactggaaaaccagagttcaccaat

SEQ ID NO: 36 - DNA, 30 bp, artificial series
  source 1..30: mol_type = other DNA
ctgaaagtgtatcacgatattaaggacatc

SEQ ID NO: 37 - DNA, 29 bp, artificial series
  source 1..29: mol_type = other DNA
acagcacggaaagaaatcattgagaacgc

SEQ ID NO: 38 - DNA, 28 bp, artificial series
  source 1..28: mol_type = other DNA
cgaactgctggatcagattgctaagatc

SEQ ID NO: 39 - DNA, 30 bp, artificial series
  source 1..30: mol_type = other DNA
ctgactatctaccagagttccgaggacatc

SEQ ID NO: 40 - DNA, 29 bp, artificial series
  source 1..29: mol_type = other DNA
caggaagagctgactaacctgaacagcga

SEQ ID NO: 41 - DNA, 28 bp, artificial series
  source 1..28: mol_type = other DNA
gctgacccaggaagagatcgaacagatt

SEQ ID NO: 42 - DNA, 30 bp, artificial series
  source 1..30: mol_type = other DNA
agtaatctgaaggggtacaccggaacacac

SEQ ID NO: 43 - DNA, 29 bp, artificial series
  source 1..29: mol_type = other DNA
aacctgtccctgaaagctatcaatctgat

SEQ ID NO: 44 - DNA, 29 bp, artificial series
  source 1..29: mol_type = other DNA
tctggatgagctgtggcatacaaacgaca

SEQ ID NO: 45 - DNA, 29 bp, artificial series
  source 1..29: mol_type = other DNA
atcagattgcaatctttaaccggctgaag

SEQ ID NO: 46 - DNA, 29 bp, artificial series
  source 1..29: mol_type = other DNA
ctggtaccaaaaaaggtggacctgagtca

SEQ ID NO: 47 - DNA, 29 bp, artificial series
  source 1..29: mol_type = other DNA
gcagaaagagatcccaaccacactggtgg

SEQ ID NO: 48 - DNA, 29 bp, artificial series
  source 1..29: mol_type = other DNA
acgatttcattctgtcacccgtggtcaag

SEQ ID NO: 49 - DNA, 29 bp, artificial series
  source 1..29: mol_type = other DNA
cggagcttcatccagagcatcaaagtgat

SEQ ID NO: 50 - DNA, 28 bp, artificial series
  source 1..28: mol_type = other DNA
caacgccatcatcaagaagtacggcctg

SEQ ID NO: 51 - DNA, 29 bp, artificial series
  source 1..29: mol_type = other DNA
cccaatgatatcattatcgagctggctag

SEQ ID NO: 52 - DNA, 30 bp, artificial series
  source 1..30: mol_type = other DNA
ggagaagaacagcaaggacgcacagaagat

SEQ ID NO: 53 - DNA, 29 bp, artificial series
  source 1..29: mol_type = other DNA
gatcaatgagatgcagaaacgaaaccggc

SEQ ID NO: 54 - DNA, 29 bp, artificial series
  source 1..29: mol_type = other DNA
agaccaatgaacgcattgaagagattatc

SEQ ID NO: 55 - DNA, 29 bp, artificial series
  source 1..29: mol_type = other DNA
cgaactaccgggaaagagaacgcaaagta

SEQ ID NO: 56 - DNA, 29 bp, artificial series
  source 1..29: mol_type = other DNA
cctgattgaaaaaatcaagctgcacgata

SEQ ID NO: 57 - DNA, 29 bp, artificial series
  source 1..29: mol_type = other DNA
tgcaggagggaaagtgtctgtattctctg

SEQ ID NO: 58 - DNA, 29 bp, artificial series
  source 1..29: mol_type = other DNA
gaggccatccccctggaggacctgctgaa

SEQ ID NO: 59 - DNA, 29 bp, artificial series
  source 1..29: mol_type = other DNA
caatccattcaactacgaggtcgatcata

SEQ ID NO: 60 - DNA, 28 bp, artificial series
  source 1..28: mol_type = other DNA
ttatccccagaagcgtgtccttcgacaa

SEQ ID NO: 61 - DNA, 30 bp, artificial series
  source 1..30: mol_type = other DNA
ttcctttaacaacaaggtgctggtcaagca

SEQ ID NO: 62 - DNA, 29 bp, artificial series
  source 1..29: mol_type = other DNA
ggaagagaactctaaaaagggcaatagga

SEQ ID NO: 63 - DNA, 28 bp, artificial series
  source 1..28: mol_type = other DNA
ctcctttccagtacctgtctagttcaga

SEQ ID NO: 64 - DNA, 30 bp, artificial series
  source 1..30: mol_type = other DNA
ttccaagatctcttacgaaacctttaaaaa

SEQ ID NO: 65 - DNA, 29 bp, artificial series
  source 1..29: mol_type = other DNA
gcacattctgaatctggccaaaggaaagg

SEQ ID NO: 66 - DNA, 29 bp, artificial series
  source 1..29: mol_type = other DNA
tccagccccagaatgtagttccttttcat

SEQ ID NO: 67 - DNA, 29 bp, artificial series
  source 1..29: mol_type = other DNA
tcccataccccacgcttgtaatcccgatg

SEQ ID NO: 68 - DNA, 29 bp, artificial series
  source 1..29: mol_type = other DNA
gatcacgtcccttgtttcatagtcaataa

SEQ ID NO: 69 - DNA, 29 bp, artificial series
  source 1..29: mol_type = other DNA
gcctccttgaacagtctgacgcctgcgtc

SEQ ID NO: 70 - DNA, 29 bp, artificial series
  source 1..29: mol_type = other DNA
ttctccgtccctcattgttttccacgttg

SEQ ID NO: 71 - DNA, 29 bp, artificial series
  source 1..29: mol_type = other DNA
tcgtttcaggcgcctggctcccctcttgc

SEQ ID NO: 72 - DNA, 29 bp, artificial series
  source 1..29: mol_type = other DNA
ttcaccctctggattctgtgccttctccg

SEQ ID NO: 73 - DNA, 29 bp, artificial series
  source 1..29: mol_type = other DNA
tcagcaggttgtaatcgaacagcagtttc

SEQ ID NO: 74 - DNA, 29 bp, artificial series
  source 1..29: mol_type = other DNA
attaattccactcagctcagaatggtcgg

SEQ ID NO: 75 - DNA, 29 bp, artificial series
  source 1..29: mol_type = other DNA
ctcaggcctttcaccctggcttcataagg

SEQ ID NO: 76 - DNA, 29 bp, artificial series
  source 1..29: mol_type = other DNA
cggaaaactcttcctctgacagcttctga

SEQ ID NO: 77 - DNA, 29 bp, artificial series
  source 1..29: mol_type = other DNA
tcggcgcttagccaggtgcagcagagctg

SEQ ID NO: 78 - DNA, 29 bp, artificial series
  source 1..29: mol_type = other DNA
tcttccacctcattgacgttatgcactcc

SEQ ID NO: 79 - DNA, 29 bp, artificial series
  source 1..29: mol_type = other DNA
cctttgtagacagctcgttgccggtgtcc

SEQ ID NO: 80 - DNA, 29 bp, artificial series
  source 1..29: mol_type = other DNA
cagagctttgctattgcgtgagatctgtt

SEQ ID NO: 81 - DNA, 29 bp, artificial series
  source 1..29: mol_type = other DNA
agctgtagctctgcgacatacttctcttc

SEQ ID NO: 82 - DNA, 29 bp, artificial series
  source 1..29: mol_type = other DNA
tcacctcgccatctttcttcagccgttcc

SEQ ID NO: 83 - DNA, 29 bp, artificial series
  source 1..29: mol_type = other DNA
gcttgtcttgaacctattaattgaccctc

SEQ ID NO: 84 - DNA, 29 bp, artificial series
  source 1..29: mol_type = other DNA
agcagctgcttggcttctttgacgtagtc

SEQ ID NO: 85 - DNA, 29 bp, artificial series
  source 1..29: mol_type = other DNA
ccagctggtggtaagccttctgcactttc

SEQ ID NO: 86 - DNA, 29 bp, artificial series
  source 1..29: mol_type = other DNA
gtcgatataagtatcgatgaagctctgat

SEQ ID NO: 87 - DNA, 29 bp, artificial series
  source 1..29: mol_type = other DNA
tcatagtaggttctccgagtctccagcag

SEQ ID NO: 88 - DNA, 29 bp, artificial series
  source 1..29: mol_type = other DNA
atccgaaggggctcccttctcctggtccc

SEQ ID NO: 89 - DNA, 29 bp, artificial series
  source 1..29: mol_type = other DNA
catctcgtaccattccttgatgtctttcc

SEQ ID NO: 90 - DNA, 29 bp, artificial series
  source 1..29: mol_type = other DNA
tctggaaaataggtgcaatgtcccatcag

SEQ ID NO: 91 - DNA, 29 bp, artificial series
  source 1..29: mol_type = other DNA
tataagcgtacttgacgcttctcagctct

SEQ ID NO: 92 - DNA, 29 bp, artificial series
  source 1..29: mol_type = other DNA
gtcattcagggcgttgtacagatctgcgt

SEQ ID NO: 93 - DNA, 29 bp, artificial series
  source 1..29: mol_type = other DNA
tcatccctggtgatgaccaggttgttcag

SEQ ID NO: 94 - DNA, 29 bp, artificial series
  source 1..29: mol_type = other DNA
acttctcatagtattccagtttctcgttt

SEQ ID NO: 95 - DNA, 29 bp, artificial series
  source 1..29: mol_type = other DNA
ctgcttaaacacgttttcgatgatctgga

SEQ ID NO: 96 - DNA, 29 bp, artificial series
  source 1..29: mol_type = other DNA
gcaatctgtttcagtgtaggctttttctt

SEQ ID NO: 97 - DNA, 29 bp, artificial series
  source 1..29: mol_type = other DNA
tgtcctcttcgttgaccaggatctcctta

SEQ ID NO: 98 - DNA, 29 bp, artificial series
  source 1..29: mol_type = other DNA
tccagtgcttgtcacccggtagcccttga

SEQ ID NO: 99 - DNA, 29 bp, artificial series
  source 1..29: mol_type = other DNA
tacactttcagattggtgaactctggttt

SEQ ID NO: 100 - DNA, 29 bp, artificial series
  source 1..29: mol_type = other DNA
tccgtgctgtgatgtccttaatatcgtga

SEQ ID NO: 101 - DNA, 29 bp, artificial series
  source 1..29: mol_type = other DNA
cagcagttcggcgttctcaatgatttctt

SEQ ID NO: 102 - DNA, 29 bp, artificial series
  source 1..29: mol_type = other DNA
tagatagtcaggatcttagcaatctgatc

SEQ ID NO: 103 - DNA, 29 bp, artificial series
  source 1..29: mol_type = other DNA
gctcttcctggatgtcctcggaactctgg

SEQ ID NO: 104 - DNA, 29 bp, artificial series
  source 1..29: mol_type = other DNA
ctgggtcagctcgctgttcaggttagtca

SEQ ID NO: 105 - DNA, 29 bp, artificial series
  source 1..29: mol_type = other DNA
ttcagattactaatctgttcgatctcttc

SEQ ID NO: 106 - DNA, 29 bp, artificial series
  source 1..29: mol_type = other DNA
gggacaggttgtgtgttccggtgtacccc

SEQ ID NO: 107 - DNA, 29 bp, artificial series
  source 1..29: mol_type = other DNA
ctcatccagaatcagattgatagctttca

SEQ ID NO: 108 - DNA, 29 bp, artificial series
  source 1..29: mol_type = other DNA
gcaatctgattgtcgtttgtatgccacag

SEQ ID NO: 109 - DNA, 29 bp, artificial series
  source 1..29: mol_type = other DNA
ttggtaccagcttcagccggttaaagatt

SEQ ID NO: 110 - DNA, 29 bp, artificial series
  source 1..29: mol_type = other DNA
ctctttctgctgactcaggtccacctttt

SEQ ID NO: 111 - DNA, 29 bp, artificial series
  source 1..29: mol_type = other DNA
atgaaatcgtccaccagtgtggttgggat

SEQ ID NO: 112 - DNA, 29 bp, artificial series
  source 1..29: mol_type = other DNA
tgaagctccgcttgaccacgggtgacaga

SEQ ID NO: 113 - DNA, 29 bp, artificial series
  source 1..29: mol_type = other DNA
gatggcgttgatcactttgatgctctgga

SEQ ID NO: 114 - DNA, 29 bp, artificial series
  source 1..29: mol_type = other DNA
atatcattgggcaggccgtacttcttgat

SEQ ID NO: 115 - DNA, 29 bp, artificial series
  source 1..29: mol_type = other DNA
tgttcttctccctagccagctcgataatg

SEQ ID NO: 116 - DNA, 29 bp, artificial series
  source 1..29: mol_type = other DNA
ctcattgatcatcttctgtgcgtccttgc

SEQ ID NO: 117 - DNA, 29 bp, artificial series
  source 1..29: mol_type = other DNA
tcattggtctgccggtttcgtttctgcat

SEQ ID NO: 118 - DNA, 29 bp, artificial series
  source 1..29: mol_type = other DNA
cggtagttcggataatctcttcaatgcgt

SEQ ID NO: 119 - DNA, 29 bp, artificial series
  source 1..29: mol_type = other DNA
ttcaatcaggtactttgcgttctctttcc

SEQ ID NO: 120 - DNA, 29 bp, artificial series
  source 1..29: mol_type = other DNA
ccctcctgcatatcgtgcagcttgatttt

SEQ ID NO: 121 - DNA, 29 bp, artificial series
  source 1..29: mol_type = other DNA
ggatggcctccagagaatacagacacttt

SEQ ID NO: 122 - DNA, 29 bp, artificial series
  source 1..29: mol_type = other DNA
gaatggattgttcagcaggtcctccaggg

SEQ ID NO: 123 - DNA, 29 bp, artificial series
  source 1..29: mol_type = other DNA
ctggggataatatgatcgacctcgtagtt

SEQ ID NO: 124 - DNA, 29 bp, artificial series
  source 1..29: mol_type = other DNA
tgttaaaggaattgtcgaaggacacgctt

SEQ ID NO: 125 - DNA, 29 bp, artificial series
  source 1..29: mol_type = other DNA
gttctcttcctgcttgaccagcaccttgt

SEQ ID NO: 126 - DNA, 29 bp, artificial series
  source 1..29: mol_type = other DNA
tggaaaggagtcctattgccctttttaga

SEQ ID NO: 127 - DNA, 29 bp, artificial series
  source 1..29: mol_type = other DNA
agatcttggaatctgaactagacaggtac

SEQ ID NO: 128 - DNA, 29 bp, artificial series
  source 1..29: mol_type = other DNA
cagaatgtgctttttaaaggtttcgtaag

SEQ ID NO: 129 - DNA, 29 bp, artificial series
  source 1..29: mol_type = other DNA
ctgatgcggccctttcctttggccagatt